European Patent Specification EP 4 010 006 B1, published November 15, 2023. Title: HLA-DR/CII peptide complexes for treating arthritis. Applicant: Fraunhofer-Gesellschaft zur Förderung der angewandten Forschung e.V. The sequence listing filed with the application follows.

SEQUENCE LISTING (42 sequences)

SEQ ID NO: 1 - protein, 11 aa, Homo sapiens
  CII peptide 261-271
AGFKGEQGPKG

SEQ ID NO: 2 - protein, 11 aa, Homo sapiens
  CII peptide 261-271, Lys = Xaa
  UNSURE 10: Xaa = any proteinogenic amino acids except Lys; preferably Xaa = Arg, Ala, Gly or Gln
AGFKGEQGPXG

SEQ ID NO: 3 - protein, 11 aa, Artificial Sequence
  CII peptide 261-271; Gln = Xaa
  UNSURE 7: Xaa = any proteinogenic amion acid except Gln; preferably Xaa = Ala, Arg, His or Gly
AGFKGEXGPKG

SEQ ID NO: 4 - protein, 11 aa, Artificial Sequence
  CII peptide 261-271; Glu = Xaa
  UNSURE 6: Xaa = any proteinogenic amino acid except Glu, preferably Xaa = Ala, Asp, Gln or Gly
AGFKGXQGPKG

SEQ ID NO: 5 - protein, 11 aa, Artificial Sequence
  CII peptide 261-271; Gly = Xaa
  UNSURE 5: Xaa = any proteinogenic amino acid expect Gly; preferably Xaa = Ala, Ser, Val or Leu
AGFKXEQGPKG

SEQ ID NO: 6 - protein, 11 aa, Artificial Sequence
  CII peptide 261-271; Gln = Xaa and Lys = Xaa
  UNSURE 7: Xaa = any proteinogenic amino acid expect Gln; preferably Xaa = Ala, Arg, His or Gly
  UNSURE 10: Xaa = any proteinogenic amino acid except Lys; preferably Xaa = Arg, Ala, Gly or Gln
AGFKGEXGPXG

SEQ ID NO: 7 - protein, 11 aa, Artificial Sequence
  CII peptide 261-271; Glu = Xaa and Lys = Xaa
  UNSURE 6: Xaa = any proteinogenic amino acid except Glu; preferably Xaa = Ala, Asp, Gln or Gly
  UNSURE 10: Xaa = any proteinogenic amino acid expect Lys, preferably Xaa = Arg, Ala, Gly or Gln
AGFKGXQGPXG

SEQ ID NO: 8 - protein, 11 aa, Artificial Sequence
  CII peptide 261-271; Gly = Xaa and Lys = Xaa
  UNSURE 5: Xaa = any proteinogenic amino acid except Gly; preferably Xaa = Ala, Ser, Val or Leu
AGFKXEQGPXG

SEQ ID NO: 9 - protein, 11 aa, Artificial Sequence
  CII peptide 261-271; Lys = Arg
AGFKGEQGPRG

SEQ ID NO: 10 - protein, 13 aa, Homo sapiens
  CII peptide 261-273
AGFKGEQGPKGEP

SEQ ID NO: 11 - protein, 13 aa, Artificial Sequence
  CII peptide 261-273; Lys = Xaa
  UNSURE 10: Xaa = any proteinogenic amino acid except Lys; preferably Lys = Arg, Ala, Gly or Gln
AGFKGEQGPXGEP

SEQ ID NO: 12 - protein, 13 aa, Artificial Sequence
  CII peptide 261-273; Lys = Arg
AGFKGEQGPRGEP

SEQ ID NO: 13 - protein, 15 aa, Homo sapiens
  CII peptide 259-273
GIAGFKGEQGPKGEP

SEQ ID NO: 14 - protein, 15 aa, Artificial Sequence
  CII peptide 259-273; Lys = Xaa
  UNSURE 12: Xaa = any proteinogenic amino acid; preferably Xaa = Arg, Ala, Gly or Gln
GIAGFKGEQGPXGEP

SEQ ID NO: 15 - protein, 15 aa, Artificial Sequence
  CII peptide 259-273; Lys = Arg
GIAGFKGEQGPRGEP

SEQ ID NO: 16 - protein, 275 aa, Artificial Sequence
  DR4 construct alpha-chain
MKLCILLAVVAFVGLSLGIKEEHVIIQAEFYLNPDQSGEFMFDFDGDEIFHVDMAKKETVWRLEEFGRFASFEAQGALANIAVDKANLEIMTKRSNYTPITNVPPEVTVLTNSPVELREPNVLICFIDKFTPPVVNVTWLRNGKPVTTGVSETVFLPREDHLFRKFHYLPFLPSTEDVYDCRVEHWGLDEPLLKHWEFDASGGGENLYFQGGGGSLTDTLQAETDQLEDEKSALQTEIANLLKEKEKLEFILAAHGGGGSGLNDIFEAQKIEWHE

SEQ ID NO: 17 - protein, 311 aa, Artificial Sequence
  DR4 construct beta-chain with hCII259-273 peptide
MKLCILLAVVAFVGLSLGSAWSHPQFEKGIAGFKGEQGPKGEPSGGGSLVPRGSGGGGSGDTRPRFLEQVKHECHFFNGTERVRFLDRYFYHQEEYVRFDSDVGEYRAVTELGRPDAEYWNSQKDLLEQKRAAVDTYCRHNYGVGESFTVQRRVYPEVTVYPAKTQPLQHHNLLVCSVNGFYPGSIEVRWFRNGQEEKTGVVSTGLIQNGDWTFQTLVMLETVPRSGEVYTCQVEHPSLTSPLTVEWRARSGGGENLYFQGGGGSRIARLEEKVKTLKAQNSELASTANMLREQVAQLKQKVMNHHHHHHH

SEQ ID NO: 18 - protein, 248 aa, Artificial Sequence
  Minimal DR4 construct alpha-chain
MKLCILLAVVAFVGLSLGIKEEHVIIQAEFYLNPDQSGEFMFDFDGDEIFHVDMAKKETVWRLEEFGRFASFEAQGALANIAVDKANLEIMTKRSNYTPITNVPPEVTVLTNSPVELREPNVLICFIDKFTPPVVNVTWLRNGKPVTTGVSETVFLPREDHLFRKFHYLPFLPSTEDVYDCRVEHWGLDEPLLKHWEFDASGGGGGGSLTDTLQAETDQLEDEKSALQTEIANLLKEKEKLEFILAAH

SEQ ID NO: 19 - protein, 288 aa, Artificial Sequence
  Minimal DR4 construct beta-chain with hCII259-273 peptide
MKLCILLAVVAFVGLSLGGIAGFKGEQGPKGEPSGGGSGGGGSGDTRPRFLEQVKHECHFFNGTERVRFLDRYFYHQEEYVRFDSDVGEYRAVTELGRPDAEYWNSQKDLLEQKRAAVDTYCRHNYGVGESFTVQRRVYPEVTVYPAKTQPLQHHNLLVCSVNGFYPGSIEVRWFRNGQEEKTGVVSTGLIQNGDWTFQTLVMLETVPRSGEVYTCQVEHPSLTSPLTVEWRARSGGGGGGSRIARLEEKVKTLKAQNSELASTANMLREQVAQLKQKVMNHHHHHHH

SEQ ID NO: 20 - protein, 311 aa, Artificial Sequence
  DR4 construct beta-chain with hCLIPmut
MKLCILLAVVAFVGLSLGSAWSHPQFEKPVSKARMATGALAQASGGGSLVPRGSGGGGSGDTRPRFLEQVKHECHFFNGTERVRFLDRYFYHQEEYVRFDSDVGEYRAVTELGRPDAEYWNSQKDLLEQKRAAVDTYCRHNYGVGESFTVQRRVYPEVTVYPAKTQPLQHHNLLVCSVNGFYPGSIEVRWFRNGQEEKTGVVSTGLIQNGDWTFQTLVMLETVPRSGEVYTCQVEHPSLTSPLTVEWRARSGGGENLYFQGGGGSRIARLEEKVKTLKAQNSELASTANMLREQVAQLKQKVMNHHHHHHH

SEQ ID NO: 21 - protein, 290 aa, Artificial Sequence
  Aq construct alpha-chain
MKLCILLAVVAFVGLSLGEDDIEADHVGFYGIVVYQSPGDIGQYTHEFDGDEWFYVDLDKKETVWMLPEFGQLTSFDPQGGLQNIATGKHNLGGWTKRSNFTPATNEAPQATVFPKSPVLLGQPNTLICFVDNIFPPVINITWLRNSKSVTDGVYETSFLVNRDHSFHKLSYLTFIPSDDDIYDCKVEHWGLDEPVLKHWEPEIPATMSELTETVSGGGENLYFQGGGGSLTDTLQAETDQLEDEKSALQTEIANLLKEKEKLEFILAAHGGGGSGLNDIFEAQKIEWHE

SEQ ID NO: 22 - protein, 316 aa, Artificial Sequence
  Aq construct beta-chain with rat CII259-273 peptide
MKLCILLAVVAFVGLSLGSAWSHPQFEKGIAGFKGEQGPKGETSGGGSLVPRGSGGGGSERHFVAQLKGECYFTNGTQRIRSVNRYIYNREEWVRFDSDVGEYRAVTELGRPDAEYWNSQPEILERTRAEVDTVCRHNYEGVETHTSLRRLEQPNVAISLSRTEALNHHNTLVCSVTDFYPAKIKVRWFRNGQEETVGVSSTQLIRNGDWTFQVLVMLEMTPHQGEVYTCHVEHPSLKSPITVEWRAQSESARSKSGGGENLYFQGGGGSRIARLEEKVKTLKAQNSELASTANMLREQVAQLKQKVMNHHHHHHH

SEQ ID NO: 23 - protein, 310 aa, Artificial Sequence
  Aq construct beta-chain with rat CII259-273 peptide without His-tag
MKLCILLAVVAFVGLSLGSAWSHPQFEKGIAGFKGEQGPKGETSGGGSLVPRGSGGGGSERHFVAQLKGECYFTNGTQRIRSVNRYIYNREEWVRFDSDVGEYRAVTELGRPDAEYWNSQPEILERTRAEVDTVCRHNYEGVETHTSLRRLEQPNVAISLSRTEALNHHNTLVCSVTDFYPAKIKVRWFRNGQEETVGVSSTQLIRNGDWTFQVLVMLEMTPHQGEVYTCHVEHPSLKSPITVEWRAQSESARSKSGGGENLYFQGGGGSRIARLEEKVKTLKAQNSELASTANMLREQVAQLKQKVMNH

SEQ ID NO: 24 - protein, 316 aa, Artificial Sequence
  Aq construct beta-chain with mCLIP peptide
MKLCILLAVVAFVGLSLGSAWSHPQFEKPVSQARMATPLLMRPSGGGSLVPRGSGGGGSERHFVAQLKGECYFTNGTQRIRSVNRYIYNREEWVRFDSDVGEYRAVTELGRPDAEYWNSQPEILERTRAEVDTVCRHNYEGVETHTSLRRLEQPNVAISLSRTEALNHHNTLVCSVTDFYPAKIKVRWFRNGQEETVGVSSTQLIRNGDWTFQVLVMLEMTPHQGEVYTCHVEHPSLKSPITVEWRAQSESARSKSGGGENLYFQGGGGSRIARLEEKVKTLKAQNSELASTANMLREQVAQLKQKVMNHHHHHHH

SEQ ID NO: 25 - protein, 310 aa, Artificial Sequence
  Aq construct beta-chain with mCLIP peptide without His-tag
MKLCILLAVVAFVGLSLGSAWSHPQFEKPVSQARMATPLLMRPSGGGSLVPRGSGGGGSERHFVAQLKGECYFTNGTQRIRSVNRYIYNREEWVRFDSDVGEYRAVTELGRPDAEYWNSQPEILERTRAEVDTVCRHNYEGVETHTSLRRLEQPNVAISLSRTEALNHHNTLVCSVTDFYPAKIKVRWFRNGQEETVGVSSTQLIRNGDWTFQVLVMLEMTPHQGEVYTCHVEHPSLKSPITVEWRAQSESARSKSGGGENLYFQGGGGSRIARLEEKVKTLKAQNSELASTANMLREQVAQLKQKVMNH

SEQ ID NO: 26 - protein, 40 aa, Homo sapiens
  cFos domain
LTDTLQAETDQLEDEKSALQTEIANLLKEKEKLEFILAAH

SEQ ID NO: 27 - protein, 40 aa, Homo sapiens
  cJun domain
RIARLEEKVKTLKAQNSELASTANMLREQVAQLKQKVMNH

SEQ ID NO: 28 - protein, 15 aa, Homo sapiens
  mutated human CLIP-peptide
PVSKARMATGALAQA

SEQ ID NO: 29 - protein, 15 aa, Homo sapiens
  rat CII-peptide 259-273
GIAGFKGEQGPKGET

SEQ ID NO: 30 - protein, 10 aa, Artificial Sequence
  streptavidin-tag
SAWSHPQFEK

SEQ ID NO: 31 - protein, 11 aa, Artificial Sequence
  Chondroitin-binding peptide
EKRIWFPYRRF

SEQ ID NO: 32 - protein, 11 aa, Artificial Sequence
  chondroitin-binding peptide
YKTNFRRYYRF

SEQ ID NO: 33 - protein, 11 aa, Artificial Sequence
  chondroitin-binding peptide
VLIRHFRKRYY

SEQ ID NO: 34 - protein, 20 aa, Artificial Sequence
  Histone NT tag
SGRGKQGGKARAKAKTRSSR

SEQ ID NO: 35 - protein, 12 aa, Artificial Sequence
  modified his-tag
NHNHNHNHNHNH

SEQ ID NO: 36 - protein, 19 aa, Artificial Sequence
  HAT-tag
KDHLIHNVHKEEHAHAHNK

SEQ ID NO: 37 - protein, 130 aa, Homo sapiens
MSGRGKQGGKARAKAKTRSSRAGLQFPVGRVHRLLRKGNYAERVGAGAPVYLAAVLEYLTAEILELAGNAARDNKKTRIIPRHLQLAIRNDEELNKLLGKVTIAQGGVLPNIQAVLLPKKTESHHKAKGK

SEQ ID NO: 38 - protein, 130 aa, Mus musculus
MSGRGKQGGKARAKAKTRSSRAGLQFPVGRVHRLLRKGNYSERVGAGAPVYLAAVLEYLTAEILELAGNAARDNKKTRIIPRHLQLAIRNDEELNKLLGRVTIAQGGVLPNIQAVLLPKKTESHHKAKGK

SEQ ID NO: 39 - protein, 30 aa, Artificial Sequence
  hCII259-273 with N-terminal and C-terminal sequence
SAWSHPQFEKGIAGFKGEQGPKGEPSGGGS

SEQ ID NO: 40 - protein, 6 aa, Artificial Sequence
  H2AC tag
HKAKGK

SEQ ID NO: 41 - protein, 6 aa, Artificial Sequence
  6XHis
HHHHHH

SEQ ID NO: 42 - protein, 7 aa, Artificial Sequence
  7xHis
HHHHHHH